European Patent Application EP 4 435 108 A1, published September 25, 2024. Title: MICROORGANISMS FOR PRODUCING L-ISOLEUCINE AND PROCESS FOR PRODUCING L-ISOLEUCINE USING THE SAME. Applicant: CJ CheilJedang Corporation. The sequence listing filed with the application follows.

SEQUENCE LISTING (31 sequences)

SEQ ID NO: 1 - protein, 424 aa, Bacillus subtilis
MSAKQVSKDEEKEALNLFLSTQTIIKEALRKLGYPGDMYELMKEPQRMLTVRIPVKMDNGSVKVFTGYRSQHNDAVGPTKGGVRFHPEVNEEEVKALSIWMTLKCGIANLPYGGGKGGIICDPRTMSFGELERLSRGYVRAISQIVGPTKDIPAPDVYTNSQIMAWMMDEYSRLREFDSPGFITGKPLVLGGSQGRETATAQGVTICIEEAVKKKGIKLQNARIIIQGFGNAGSFLAKFMHDAGAKVIGISDANGGLYNPDGLDIPYLLDKRDSFGMVTNLFTDVITNEELLEKDCDILVPAAISNQITAKNAHNIQASIVVEAANGPTTIDATKILNERGVLLVPDILASAGGVTVSYFEWVQNNQGYYWSEEEVAEKLRSVMVSSFETIYQTAATHKVDMRLAAYMTGIRKSAEASRFRGWV

SEQ ID NO: 2 - DNA, 1275 bp, Bacillus subtilis
  source 1..1275: mol_type = genomic DNA
atgtcagcaaagcaagtctcgaaagatgaagaaaaagaagctcttaacttatttctgtctacccaaacaatcattaaggaagcccttcggaagctgggttatccgggagatatgtatgaactcatgaaagagccgcagagaatgctcactgtccgcattccggtcaaaatggacaatgggagcgtcaaagtgttcacaggctaccggtcacagcacaatgatgctgtcggtccgacaaaggggggcgttcgcttccatccagaagttaatgaagaggaagtaaaggcattatccatttggatgacgctcaaatgcgggattgccaatcttccttacggcggcgggaagggcggtattatttgtgatccgcggacaatgtcatttggagaactggaaaggctgagcagggggtatgtccgtgccatcagccagatcgtcggtccgacaaaggatattccagctcccgatgtgtacaccaattcgcagattatggcgtggatgatggatgagtacagccggctgcgggaattcgattctccgggctttattacaggtaaaccgcttgttttgggaggatcgcaaggacgggaaacagcgacggcacagggcgtcacgatttgtattgaagaggcggtgaagaaaaaagggatcaagctgcaaaacgcgcgcatcatcatacagggctttggaaacgcgggtagcttcctggccaaattcatgcacgatgcgggcgcgaaggtgatcgggatttctgatgccaatggcgggctctacaacccagacggccttgatatcccttatttgctcgataaacgggacagctttggtatggtcaccaatttatttactgacgtcatcacaaatgaggagctgcttgaaaaggattgcgatattttagtgcctgccgcgatctccaatcaaatcacagccaaaaacgcacataacattcaggcgtcaatcgtcgttgaagcggcgaacggcccgacaaccattgatgccactaagatcctgaatgaaagaggcgtgctgcttgtgccggatatcctagcgagtgccggcggcgtcacggtttcttattttgaatgggtgcaaaacaaccaaggatattattggtcggaagaagaggttgcagaaaaactgagaagcgtcatggtcagctcgttcgaaacaatttatcaaacagcggcaacacataaagtggatatgcgtttggcggcttacatgacgggcatcagaaaatcggcagaagcatcgcgtttccgcggatgggtctaa

SEQ ID NO: 3 - protein, 461 aa, unidentified
  REGION 1..461: note = Rhodospirillales
MSKSHSGAKTQEYLERYMEGVTKRNPGQPEFVQAVYEVASTIFPYISDKPQYHENQILERMAEPERVISFRVPWTDDSGNIRTNRGWRVQFNSAIGPYKGLRFHPSVNLGIIKFLGFEQIFKNSLTTLAMGGGKGGSDFDPKGKSDLEVMKFTQSFMRELFRHIGADVDVPAGDIGVGGREIGFLYGYYKKIRNEFTGVLTGRALEFGGSLIRPEATGYGAVYFGAEMLATRKKDYKGLRCLVSGKGNVTQYTIEKINQLGGKAISISDSGGTIIDEDGISAERLNYVMELENVRRGRAKEYAEKYKSAKYYEGKSVWDVVKDEGLQFDCAFPSATQNEIDEQHATAMVKNGCFLVSEGANMPSNLAAIKVYQGANILYGPAKAANAGGVAVSGLEMAQQSARWYWSREEVDQKLHRIMQAIHKQCLDASKAYATEGDYLAGANIAGFIKVAHAMVAEGVV

SEQ ID NO: 4 - DNA, 1386 bp, unidentified
  misc_feature 1..1386: note = Rhodospirillales
  source 1..1386: mol_type = genomic DNA
atgtctaaaagccacagcggcgctaaaacccaggaatatctggaacgttacatggaaggtgttaccaaacgtaatccgggccagccggaatttgttcaggcagtttatgaagttgctagcaccatcttcccgtacatttctgataaaccgcagtaccatgaaaaccagatcctggaacgtatggctgaaccggaacgcgttatctccttccgtgttccgtggaccgatgactctggtaatattcgtaccaaccgtggttggcgtgtgcagttcaactccgcgatcggcccgtacaaaggtctgcgtttccacccgtctgtgaacctgggtatcatcaaattcctgggcttcgaacagatctttaaaaactccctgaccaccctggctatgggcggtggcaaaggtggcagcgactttgatccgaaaggcaaaagcgatctggaagttatgaaattcacccagtcgtttatgcgcgaactgttccgtcacattggcgcggatgttgatgttccggcgggtgatatcggtgttggtggccgtgaaatcggcttcctgtacggctattataagaaaatccgtaatgaatttaccggtgtgctgaccggccgtgctctggaattcggtggcagcctgatccgtccggaagcgaccggctacggcgcggtttattttggcgcagaaatgctggccacccgtaaaaaagactataaaggcctgcgttgcctggtttctggtaaaggcaacgtcacccagtacaccattgaaaaaattaaccagctgggcggcaaagctatctctatctccgactctggcggtaccattatcgatgaagatggcatttctgcagaacgtctgaactatgtaatggaactggaaaacgttcgtcgcggccgtgcaaaagaatacgctgaaaaatataaatctgcgaaatattacgaaggtaaatccgtttgggacgttgttaaggacgaaggtctgcagttcgattgcgcgttcccgtctgcaacccagaacgaaatcgatgaacagcacgcaaccgcgatggtgaaaaacggctgcttcctggttagcgaaggtgcgaacatgccgtccaacctggcagcgattaaagtttaccagggtgctaacattctgtacggtccggctaaagcagcaaacgcaggtggtgttgcggttagcggtctggaaatggctcagcagagcgcgcgttggtactggtctcgtgaagaagttgatcaaaaattacaccgtattatgcaggcaattcataaacagtgtttagacgcttctaaagcgtacgcgaccgaaggtgattatctggcgggtgctaacattgctggttttattaaagttgcgcacgccatggttgcggaaggtgtggtttaa

SEQ ID NO: 5 - DNA, 35 bp, synthetic construct
  misc_feature 1..35: note = primer
  source 1..35: mol_type = other DNA
tgaattcgagctcggtacccaggcgcagggccggg

SEQ ID NO: 6 - DNA, 21 bp, synthetic construct
  misc_feature 1..21: note = primer
  source 1..21: mol_type = other DNA
gggcaacgcccacacgcagcg

SEQ ID NO: 7 - DNA, 21 bp, synthetic construct
  misc_feature 1..21: note = primer
  source 1..21: mol_type = other DNA
aggggccccgctgaagtcatc

SEQ ID NO: 8 - DNA, 35 bp, synthetic construct
  misc_feature 1..35: note = primer
  source 1..35: mol_type = other DNA
gactctagaggatccccgcagatccagtccatccc

SEQ ID NO: 9 - DNA, 39 bp, synthetic construct
  misc_feature 1..39: note = primer
  source 1..39: mol_type = other DNA
ctgcgtgtgggcgttgccctaccaattccatttgagggc

SEQ ID NO: 10 - DNA, 16 bp, synthetic construct
  misc_feature 1..16: note = primer
  source 1..16: mol_type = other DNA
gatttcctcgttccca

SEQ ID NO: 11 - DNA, 39 bp, synthetic construct
  misc_feature 1..39: note = primer
  source 1..39: mol_type = other DNA
atgacttcagcggggccccttagatgacgccctgtgcca

SEQ ID NO: 12 - DNA, 38 bp, synthetic construct
  misc_feature 1..38: note = primer
  source 1..38: mol_type = other DNA
gatgggaacgaggaaatcatggatcagacatattctct

SEQ ID NO: 13 - DNA, 39 bp, synthetic construct
  misc_feature 1..39: note = primer
  source 1..39: mol_type = other DNA
gatgacttcagcggggccccttaaatcacaccctgcgcc

SEQ ID NO: 14 - DNA, 38 bp, synthetic construct
  misc_feature 1..38: note = primer
  source 1..38: mol_type = other DNA
gatgggaacgaggaaatcatgtcagcaaagcaagtctc

SEQ ID NO: 15 - DNA, 38 bp, synthetic construct
  misc_feature 1..38: note = primer
  source 1..38: mol_type = other DNA
gatgacttcagcggggccccttagacccatccgcggaa

SEQ ID NO: 16 - DNA, 38 bp, synthetic construct
  misc_feature 1..38: note = primer
  source 1..38: mol_type = other DNA
gatgggaacgaggaaatcatgtctaaaagccacagcgg

SEQ ID NO: 17 - DNA, 38 bp, synthetic construct
  misc_feature 1..38: note = primer
  source 1..38: mol_type = other DNA
gatgacttcagcggggccccttaaaccacaccttccgc

SEQ ID NO: 18 - DNA, 38 bp, synthetic construct
  misc_feature 1..38: note = primer
  source 1..38: mol_type = other DNA
gatgggaacgaggaaatcatgagcgaactacaccccaa

SEQ ID NO: 19 - DNA, 39 bp, synthetic construct
  misc_feature 1..39: note = primer
  source 1..39: mol_type = other DNA
gatgacttcagcggggcccctcagatgagcccgagtgcg

SEQ ID NO: 20 - DNA, 1338 bp, synthetic construct
  misc_feature 1..1338: note = R407H
  source 1..1338: mol_type = other DNA
atgacctcagcatctgccccaagctttaaccccggcaagggtcccggctcagcagtcggaattgcccttttaggattcggaacagtcggcactgaggtgatgcgtctgatgaccgagtacggtgatgaacttgcgcaccgcattggtggcccactggaggttcgtggcattgctgtttctgatatctcaaagccacgtgaaggcgttgcacctgagctgctcactgaggacgcttttgcactcatcgagcgcgaggatgttgacatcgtcgttgaggttatcggcggcattgagtacccacgtgaggtagttctcgcagctctgaaggccggcaagtctgttgttaccgccaataaggctcttgttgcagctcactctgctgagcttgctgatgcagcggaagccgcaaacgttgacctgtacttcgaggctgctgttgcaggcgcaattccagtggttggcccactgcgtcgctccctggctggcgatcagatccagtctgtgatgggcatcgttaacggcaccaccaacttcatcttggacgccatggattccaccggcgctgactatgcagattctttggctgaggcaactcgtttgggttacgccgaagctgatccaactgcagacgtcgaaggccatgacgccgcatccaaggctgcaattttggcatccatcgctttccacacccgtgttaccgcggatgatgtgtactgcgaaggtatcagcaacatcagcgctgccgacattgaggcagcacagcaggcaggccacaccatcaagttgttggccatctgtgagaagttcaccaacaaggaaggaaagtcggctatttctgctcgcgtgcacccgactctattacctgtgtcccacccactggcgtcggtaaacaagtcctttaatgcaatctttgttgaagcagaagcagctggtcgcctgatgttctacggaaacggtgcaggtggcgcgccaaccgcgtctgctgtgcttggcgacgtcgttggtgccgcacgaaacaaggtgcacggtggccgtgctccaggtgagtccacctacgctaacctgccgatcgctgatttcggtgagaccaccactcgttaccacctcgacatggatgtggaagatcgcgtgggggttttggctgaattggctagcctgttctctgagcaaggaatctccctgcgtacaatccgacaggaagagcgcgatgatgatgcacatctgatcgtggtcacccactctgcgctggaatctgatctttcccgcaccgttgaactgctgaaggctaagcctgttgttaaggcaatcaacagtgtgatccgcctcgaaagggactaa

SEQ ID NO: 21 - DNA, 35 bp, synthetic construct
  misc_feature 1..35: note = primer
  source 1..35: mol_type = other DNA
tcgagctcggtaccccgcttttgcactcatcgagc

SEQ ID NO: 22 - DNA, 23 bp, synthetic construct
  misc_feature 1..23: note = primer
  source 1..23: mol_type = other DNA
cacgatcagatgtgcatcatcat

SEQ ID NO: 23 - DNA, 23 bp, synthetic construct
  misc_feature 1..23: note = primer
  source 1..23: mol_type = other DNA
atgatgatgcacatctgatcgtg

SEQ ID NO: 24 - DNA, 35 bp, synthetic construct
  misc_feature 1..35: note = primer
  source 1..35: mol_type = other DNA
ctctagaggatccccgagcatcttccaaaaccttg

SEQ ID NO: 25 - protein, 436 aa, Corynebacterium glutamicum
MSETYVSEKSPGVMASGAELIRAADIQTAQARISSVIAPTPLQYCPRLSEETGAEIYLKREDLQDVRSYKIRGALNSGAQLTQEQRDAGIVAASAGNHAQGVAYVCKSLGVQGRIYVPVQTPKQKRDRIMVHGGEFVSLVVTGNNFDEASAAAHEDAERTGATLIEPFDARNTVIGQGTVAAEILSQLTSMGKSADHVMVPVGGGGLLAGVVSYMADMAPRTAIVGIEPAGAASMQAALHNGGPITLETVDPFVDGAAVKRVGDLNYTIVEKNQGRVHMMSATEGAVCTEMLDLYQNEGIIAEPAGALSIAGLKEMSFAPGSVVVCIISGGNNDVLRYAEIAERSLVHRGLKHYFLVNFPQKPGQLRHFLEDILGPDDDITLFEYLKRNNRETGTALVGIHLSEASGLDSLLERMEESAIDSRRLEPGTPEYEYLT

SEQ ID NO: 26 - DNA, 35 bp, synthetic construct
  misc_feature 1..35: note = primer
  source 1..35: mol_type = other DNA
tcgagctcggtacccatgagtgaaacatacgtgtc

SEQ ID NO: 27 - DNA, 39 bp, synthetic construct
  misc_feature 1..39: note = primer
  source 1..39: mol_type = other DNA
gcgcttgaggtactctgccagcgcgatgtcatcatccgg

SEQ ID NO: 28 - DNA, 39 bp, synthetic construct
  misc_feature 1..39: note = primer
  source 1..39: mol_type = other DNA
ccggatgatgacatcgcgctggcagagtacctcaagcgc

SEQ ID NO: 29 - DNA, 34 bp, synthetic construct
  misc_feature 1..34: note = primer
  source 1..34: mol_type = other DNA
ctctagaggatcccccgtcaccgacacctccaca

SEQ ID NO: 30 - DNA, 20 bp, synthetic construct
  misc_feature 1..20: note = primer
  source 1..20: mol_type = other DNA
aactgatgcctgaggacaag

SEQ ID NO: 31 - DNA, 20 bp, synthetic construct
  misc_feature 1..20: note = primer
  source 1..20: mol_type = other DNA
gcttgataccgaagcaaacc